European Patent Specification EP 3 747 454 B9, published October 4, 2023. Title: AMYLOID-BETA-BINDING PEPTIDES AND THE USE THEREOF FOR THE TREATMENT AND DIAGNOSIS OF ALZHEIMER'S DISEASE. Applicant: Forschungszentrum Juelich GmbH. The sequence listing filed with the application follows.

SEQUENCE LISTING (12 sequences)

SEQ ID NO: 1 - protein, 12 aa, Artificial Sequence
  D-Peptide, RD2
PTLHTHNRRRRR

SEQ ID NO: 2 - protein, 12 aa, Artificial Sequence
  D-Peptide, D3
RPRTRLHTHRNR

SEQ ID NO: 3 - protein, 12 aa, Artificial Sequence
  D-Peptide, DB3
RPITRLRTHQNR

SEQ ID NO: 4 - protein, 24 aa, Artificial Sequence
  D-Peptide, RD2D3
PTLHTHNRRRRRRPRTRLHTHRNR

SEQ ID NO: 5 - protein, 24 aa, Artificial Sequence
  D-Peptide, D3RD2
RPRTRLHTHRNRPTLHTHNRRRRR

SEQ ID NO: 6 - protein, 24 aa, Artificial Sequence
  D-Peptide, D3D3
RPRTRLHTHRNRRPRTRLHTHRNR

SEQ ID NO: 7 - protein, 24 aa, Artificial Sequence
  D-Peptide, RD2RD2
PTLHTHNRRRRRPTLHTHNRRRRR

SEQ ID NO: 8 - protein, 24 aa, Artificial Sequence
  D-Peptide, DB3DB3
RPITRLRTHQNRRPITRLRTHQNR

SEQ ID NO: 9 - protein, 13 aa, Artificial Sequence
  D-Peptide, D3r
RPRTRLHTHRNRR

SEQ ID NO: 10 - protein, 13 aa, Artificial Sequence
  D-Peptide, D3p
RPRTRLHTHRNRP

SEQ ID NO: 11 - protein, 13 aa, Artificial Sequence
  D-Peptide, D3a
RPRTRLHTHRNRA

SEQ ID NO: 12 - protein, 12 aa, Artificial Sequence
  D-Peptide, D3(p2k)
RKRTRLHTHRNR